European Patent Application EP 4 603 585 A1, published August 20, 2025. Title: SNRNA NUCLEIC ACID MOLECULE AND APPLICATION THEREOF. Applicant: GUANGZHOU REFORGENE MEDICINE CO., LTD. The sequence listing filed with the application follows.

SEQUENCE LISTING (82 sequences)

SEQ ID NO: 1 - RNA, 684 nt, synthetic construct
  source 1..684: mol_type = other RNA
taaatatattttatctttagggcttaggtgtgatcattgcaattttggatttaaatttctccgaagctttaatgatgttggatgtgagccctgccagtgtaacctccatggctcagtgaacaaattctgcaatcctcactctgggcagtgtgagtgcaaaaaagaagccaaaggacttcagtgtgacacctgcagagaaaacttttatgggttagatgtcaccaattgtaaggcctgtgactgtgacacagctggatccctccctgggactgtctgtaatgctaagacagggcagtgcatctgcaagcccaatgttgaagggagacagtgcaataaatgtttggagggaaacttctacctacggcaaaataattctttcctctgtctgccttgcaactgtgataagactgggacaataaatggctctctgctgtgtaacaaatcaacaggacaatgtccttgcaaattaggggtaacaggtcttcgctgtaatcagtgtgagcctcacaggtacaatttgaccattgacaattttcaacactgccagatgtgtgagtgtgattccttggggacattacctgggaccatttgtgacccaatcagtggccagtgcctgtgtgtgcctaatcgtcaaggaagaaggtgtaatcagtgtcaaccaggtaagaaagaaatgtattacat

SEQ ID NO: 2 - RNA, 117 nt, synthetic construct
  source 1..117: mol_type = other RNA
taaatatattttatctttagggcttaggtgtgatcattgcaattttggatttaaatttctccgaagctttaatgatgttggatgtgagccctgccagtgtaacctccatggctcagt

SEQ ID NO: 3 - RNA, 191 nt, synthetic construct
  source 1..191: mol_type = other RNA
cagtgtgagcctcacaggtacaatttgaccattgacaattttcaacactgccagatgtgtgagtgtgattccttggggacattacctgggaccatttgtgacccaatcagtggccagtgcctgtgtgtgcctaatcgtcaaggaagaaggtgtaatcagtgtcaaccaggtaagaaagaaatgtattacat

SEQ ID NO: 4 - RNA, 87 nt, synthetic construct
  source 1..87: mol_type = other RNA
aatcagtggccagtgcctgtgtgtgcctaatcgtcaaggaagaaggtgtaatcagtgtcaaccaggtaagaaagaaatgtattacat

SEQ ID NO: 5 - RNA, 11 nt, synthetic construct
  source 1..11: mol_type = other RNA
aatttgtctag

SEQ ID NO: 6 - RNA, 11 nt, synthetic construct
  source 1..11: mol_type = other RNA
aatttttggag

SEQ ID NO: 7 - RNA, 31 nt, synthetic construct
  source 1..31: mol_type = other RNA
caggttttctgacttcggtcggaaaacccct

SEQ ID NO: 8 - DNA, 13 bp, synthetic construct
  source 1..13: mol_type = other DNA
gtctacaatgaaa

SEQ ID NO: 9 - RNA, 64 nt, synthetic construct
  source 1..64: mol_type = other RNA
tgcctaatcgtcaaggaagaaggtgtaatcagtgtcaaccaggtaagaaagaaatgtattacat

SEQ ID NO: 10 - RNA, 64 nt, synthetic construct
  source 1..64: mol_type = other RNA
tgcctaatcgtcaaggaagaaggtgtaatcagtggcaaccaggtaagaaagaaatgtattacat

SEQ ID NO: 11 - RNA, 24 nt, synthetic construct
  source 1..24: mol_type = other RNA
attgtacctgtgaggctcacactg

SEQ ID NO: 12 - RNA, 24 nt, synthetic construct
  source 1..24: mol_type = other RNA
accttcttccttgacgattaggca

SEQ ID NO: 13 - RNA, 24 nt, synthetic construct
  source 1..24: mol_type = other RNA
attacaccttcttccttgacgatt

SEQ ID NO: 14 - RNA, 27 nt, synthetic construct
  source 1..27: mol_type = other RNA
attacaccttcttccttgacgattagg

SEQ ID NO: 15 - RNA, 24 nt, synthetic construct
  source 1..24: mol_type = other RNA
actgattacaccttcttccttgac

SEQ ID NO: 16 - RNA, 24 nt, synthetic construct
  source 1..24: mol_type = other RNA
acatttctttcttacctggttgac

SEQ ID NO: 17 - RNA, 22 nt, synthetic construct
  source 1..22: mol_type = other RNA
acatttctttcttacctggttg

SEQ ID NO: 18 - RNA, 27 nt, synthetic construct
  source 1..27: mol_type = other RNA
acatttctttcttacctggttgacact

SEQ ID NO: 19 - RNA, 24 nt, synthetic construct
  source 1..24: mol_type = other RNA
acatttctttcttacctggttgcc

SEQ ID NO: 20 - RNA, 27 nt, synthetic construct
  source 1..27: mol_type = other RNA
acatttctttcttacctggttgccact

SEQ ID NO: 21 - RNA, 24 nt, synthetic construct
  source 1..24: mol_type = other RNA
aatacatttctttcttacctggtt

SEQ ID NO: 22 - RNA, 24 nt, synthetic construct
  source 1..24: mol_type = other RNA
atgtaatacatttctttcttacct

SEQ ID NO: 23 - RNA, 20 nt, synthetic construct
  source 1..20: mol_type = other RNA
aggtgtagtcgaccatcgtg

SEQ ID NO: 24 - RNA, 66 nt, synthetic construct
  source 1..66: mol_type = other RNA
  modified_base 1: mod_base = OTHER; note = 2'-OME
  modified_base 2: mod_base = um
  modified_base 3: mod_base = um
  modified_base 64: mod_base = cm
  modified_base 65: mod_base = cm
  modified_base 66: mod_base = um
  modified_base 1: mod_base = OTHER; note = phosphorothioate backbone
  modified_base 2: mod_base = OTHER; note = phosphorothioate backbone
  modified_base 3: mod_base = OTHER; note = phosphorothioate backbone
  modified_base 64: mod_base = OTHER; note = phosphorothioate backbone
  modified_base 65: mod_base = OTHER; note = phosphorothioate backbone
  modified_base 66: mod_base = OTHER; note = phosphorothioate backbone
attacaccttcttccttgacgattaatttttggagcaggttttctgacttcggtcggaaaacccct

SEQ ID NO: 25 - RNA, 75 nt, synthetic construct
  source 1..75: mol_type = other RNA
  modified_base 1: mod_base = OTHER; note = 2'-OME
  modified_base 2: mod_base = cm
  modified_base 3: mod_base = um
  modified_base 73: mod_base = cm
  modified_base 74: mod_base = cm
  modified_base 75: mod_base = um
  modified_base 1: mod_base = OTHER; note = phosphorothioate backbone
  modified_base 2: mod_base = OTHER; note = phosphorothioate backbone
  modified_base 3: mod_base = OTHER; note = phosphorothioate backbone
  modified_base 73: mod_base = OTHER; note = phosphorothioate backbone
  modified_base 74: mod_base = OTHER; note = phosphorothioate backbone
  modified_base 75: mod_base = OTHER; note = phosphorothioate backbone
actgattacaccttcttccttgacgattaggcaaatttttggagcaggttttctgacttcggtcggaaaacccct

SEQ ID NO: 26 - RNA, 69 nt, synthetic construct
  source 1..69: mol_type = other RNA
  modified_base 1: mod_base = OTHER; note = 2'-OME
  modified_base 2: mod_base = um
  modified_base 3: mod_base = um
  modified_base 67: mod_base = cm
  modified_base 68: mod_base = cm
  modified_base 69: mod_base = um
  modified_base 1: mod_base = OTHER; note = phosphorothioate backbone
  modified_base 2: mod_base = OTHER; note = phosphorothioate backbone
  modified_base 3: mod_base = OTHER; note = phosphorothioate backbone
  modified_base 67: mod_base = OTHER; note = phosphorothioate backbone
  modified_base 68: mod_base = OTHER; note = phosphorothioate backbone
  modified_base 69: mod_base = OTHER; note = phosphorothioate backbone
attacaccttcttccttgacgattaggaatttttggagcaggttttctgacttcggtcggaaaacccct

SEQ ID NO: 27 - RNA, 82 nt, synthetic construct
  source 1..82: mol_type = other RNA
  modified_base 1: mod_base = OTHER; note = 2'-OME
  modified_base 2: mod_base = um
  modified_base 3: mod_base = um
  modified_base 80: mod_base = cm
  modified_base 81: mod_base = cm
  modified_base 82: mod_base = um
  modified_base 1: mod_base = OTHER; note = phosphorothioate backbone
  modified_base 2: mod_base = OTHER; note = phosphorothioate backbone
  modified_base 3: mod_base = OTHER; note = phosphorothioate backbone
  modified_base 80: mod_base = OTHER; note = phosphorothioate backbone
  modified_base 81: mod_base = OTHER; note = phosphorothioate backbone
  modified_base 82: mod_base = OTHER; note = phosphorothioate backbone
attacaccttcttccttgacgattaggcacacacaggcacaatttttggagcaggttttctgacttcggtcggaaaacccct

SEQ ID NO: 28 - DNA, 336 bp, synthetic construct
  source 1..336: mol_type = other DNA
atggtgagcaagggcgaggagctgttcaccggggtggtgcccatcctggtcgagctggacggcgacgtaaacggccacaagttcagcgtgtccggcgagggcgagggcgatgccacctacggcaagctgaccctgaagttcatctgcaccaccggcaagctgcccgtgccctggcccaccctcgtgaccaccctgacctacggcgtgcagtgcttcagccgctaccccgaccacatgaagcagcacgacttcttcaagtccgccatgcccgaaggctacgtccaggagcgcaccatcttcttcaaggacgacggcaactacaagacccgcgccgag

SEQ ID NO: 29 - DNA, 384 bp, synthetic construct
  source 1..384: mol_type = other DNA
gtgaagttcgagggcgacaccctggtgaaccgcatcgagctgaagggcatcgacttcaaggaggacggcaacatcctggggcacaagctggagtacaactacaacagccacaacgtctatatcatggccgacaagcagaagaacggcatcaaggtgaacttcaagatccgccacaacatcgaggacggcagcgtgcagctcgccgaccactaccagcagaacacccccatcggcgacggccccgtgctgctgcccgacaaccactacctgagcacccagtccgccctgagcaaagaccccaacgagaagcgcgatcacatggtcctgctggagttcgtgaccgccgccgggatcactctcggcatggacgagctgtacaagtaa

SEQ ID NO: 30 - DNA, 21 bp, synthetic construct
  source 1..21: mol_type = other DNA
agcctttccgccaaggtgatc

SEQ ID NO: 31 - DNA, 21 bp, synthetic construct
  source 1..21: mol_type = other DNA
cacaacgttgcccagcaatgg

SEQ ID NO: 32 - RNA, 44 nt, synthetic construct
  source 1..44: mol_type = other RNA
cgaagctttaatgatgttggatgtgagccctgccagtgtaacct

SEQ ID NO: 33 - RNA, 32 nt, synthetic construct
  source 1..32: mol_type = other RNA
gagccctgccagtgtaacctccatggctcagt

SEQ ID NO: 34 - RNA, 34 nt, synthetic construct
  source 1..34: mol_type = other RNA
aatcagtggccagtgcctgtgtgtgcctaatcgt

SEQ ID NO: 35 - RNA, 20 nt, synthetic construct
  source 1..20: mol_type = other RNA
tatgatagggacttagggtg

SEQ ID NO: 36 - RNA, 37 nt, synthetic construct
  source 1..37: mol_type = other RNA
taaatatattttatctttagggcttaggtgtgatcat

SEQ ID NO: 37 - RNA, 29 nt, synthetic construct
  source 1..29: mol_type = other RNA
ctttagggcttaggtgtgatcattgcaat

SEQ ID NO: 38 - RNA, 34 nt, synthetic construct
  source 1..34: mol_type = other RNA
ggtgtgatcattgcaattttggatttaaatttct

SEQ ID NO: 39 - RNA, 34 nt, synthetic construct
  source 1..34: mol_type = other RNA
ttggatttaaatttctccgaagctttaatgatgt

SEQ ID NO: 40 - RNA, 24 nt, synthetic construct
  source 1..24: mol_type = other RNA
agccctaaagataaaatatattta

SEQ ID NO: 41 - RNA, 24 nt, synthetic construct
  source 1..24: mol_type = other RNA
acctaagccctaaagataaaatat

SEQ ID NO: 42 - RNA, 24 nt, synthetic construct
  source 1..24: mol_type = other RNA
atcacacctaagccctaaagataa

SEQ ID NO: 43 - RNA, 27 nt, synthetic construct
  source 1..27: mol_type = other RNA
atgatcacacctaagccctaaagataa

SEQ ID NO: 44 - RNA, 24 nt, synthetic construct
  source 1..24: mol_type = other RNA
aatgatcacacctaagccctaaag

SEQ ID NO: 45 - RNA, 24 nt, synthetic construct
  source 1..24: mol_type = other RNA
attgcaatgatcacacctaagccc

SEQ ID NO: 46 - RNA, 24 nt, synthetic construct
  source 1..24: mol_type = other RNA
atccaaaattgcaatgatcacacc

SEQ ID NO: 47 - RNA, 24 nt, synthetic construct
  source 1..24: mol_type = other RNA
atttaaatccaaaattgcaatgat

SEQ ID NO: 48 - RNA, 24 nt, synthetic construct
  source 1..24: mol_type = other RNA
agaaatttaaatccaaaattgcaa

SEQ ID NO: 49 - RNA, 24 nt, synthetic construct
  source 1..24: mol_type = other RNA
agcttcggagaaatttaaatccaa

SEQ ID NO: 50 - RNA, 24 nt, synthetic construct
  source 1..24: mol_type = other RNA
attaaagcttcggagaaatttaaa

SEQ ID NO: 51 - RNA, 24 nt, synthetic construct
  source 1..24: mol_type = other RNA
acatcattaaagcttcggagaaat

SEQ ID NO: 52 - RNA, 24 nt, synthetic construct
  source 1..24: mol_type = other RNA
acatccaacatcattaaagcttcg

SEQ ID NO: 53 - RNA, 24 nt, synthetic construct
  source 1..24: mol_type = other RNA
agggctcacatccaacatcattaa

SEQ ID NO: 54 - RNA, 22 nt, synthetic construct
  source 1..22: mol_type = other RNA
acactggcagggctcacatcca

SEQ ID NO: 55 - RNA, 27 nt, synthetic construct
  source 1..27: mol_type = other RNA
acactggcagggctcacatccaacatc

SEQ ID NO: 56 - RNA, 24 nt, synthetic construct
  source 1..24: mol_type = other RNA
aggttacactggcagggctcacat

SEQ ID NO: 57 - RNA, 24 nt, synthetic construct
  source 1..24: mol_type = other RNA
atggaggttacactggcagggctc

SEQ ID NO: 58 - RNA, 24 nt, synthetic construct
  source 1..24: mol_type = other RNA
actgagccatggaggttacactgg

SEQ ID NO: 59 - RNA, 24 nt, synthetic construct
  source 1..24: mol_type = other RNA
acacacaggcactggccactgatt

SEQ ID NO: 60 - RNA, 24 nt, synthetic construct
  source 1..24: mol_type = other RNA
aggcacacacaggcactggccact

SEQ ID NO: 61 - RNA, 24 nt, synthetic construct
  source 1..24: mol_type = other RNA
acgattaggcacacacaggcactg

SEQ ID NO: 62 - DNA, 437 bp, synthetic construct
  source 1..437: mol_type = other DNA
aagcttaacaacataggagctgtgattggctgttttcagccaatcagcactgactcatttgcatagcctttacaagcggtcacaaactcaagaaacgagcggttttaatagtcttttagaatattgtttatcgaaccgaataaggaactgtgctttgtgattcacatatcagtggaggggtgtggaaatggcaccttgatctcaccctcatcgaaagtggagttgatgtccttccctggctcgctacagacgcacttccgcagagaccaatgtgggtctcgaatttttggagcaggttttctgacttcggtcggaaaacccctcccaatttcactggtctacaatgaaagcaaaacagttctcttccccgctccccggtgtgtgagaggggctttgatccttctctggtttcctaggaaacgcgtatgtgcggccgc

SEQ ID NO: 63 - RNA, 90 nt, synthetic construct
  source 1..90: mol_type = other RNA
  modified_base 1: mod_base = OTHER; note = 2'-OME
  modified_base 2: mod_base = cm
  modified_base 3: mod_base = OTHER; note = 2'-OME
  modified_base 88: mod_base = cm
  modified_base 89: mod_base = cm
  modified_base 90: mod_base = um
  modified_base 1: mod_base = OTHER; note = phosphorothioate backbone
  modified_base 2: mod_base = OTHER; note = phosphorothioate backbone
  modified_base 3: mod_base = OTHER; note = phosphorothioate backbone
  modified_base 88: mod_base = OTHER; note = phosphorothioate backbone
  modified_base 89: mod_base = OTHER; note = phosphorothioate backbone
  modified_base 90: mod_base = OTHER; note = phosphorothioate backbone
acatttctttcttacctggttgacatcacacctaagccctaaagataaaatttttggagcaggttttctgacttcggtcggaaaacccct

SEQ ID NO: 64 - RNA, 97 nt, synthetic construct
  source 1..97: mol_type = other RNA
  modified_base 1: mod_base = OTHER; note = 2'-OME
  modified_base 2: mod_base = OTHER; note = 2'-OME
  modified_base 3: mod_base = cm
  modified_base 95: mod_base = cm
  modified_base 96: mod_base = cm
  modified_base 97: mod_base = um
  modified_base 1: mod_base = OTHER; note = phosphorothioate backbone
  modified_base 2: mod_base = OTHER; note = phosphorothioate backbone
  modified_base 3: mod_base = OTHER; note = phosphorothioate backbone
  modified_base 95: mod_base = OTHER; note = phosphorothioate backbone
  modified_base 96: mod_base = OTHER; note = phosphorothioate backbone
  modified_base 97: mod_base = OTHER; note = phosphorothioate backbone
aacatttctttcttacctggttgacactatgatcacacctaagccctaaagataaaatttttggagcaggttttctgacttcggtcggaaaacccct

SEQ ID NO: 65 - RNA, 88 nt, synthetic construct
  source 1..88: mol_type = other RNA
  modified_base 1: mod_base = OTHER; note = 2'-OME
  modified_base 2: mod_base = um
  modified_base 3: mod_base = um
  modified_base 86: mod_base = cm
  modified_base 87: mod_base = cm
  modified_base 88: mod_base = um
  modified_base 1: mod_base = OTHER; note = phosphorothioate backbone
  modified_base 2: mod_base = OTHER; note = phosphorothioate backbone
  modified_base 3: mod_base = OTHER; note = phosphorothioate backbone
  modified_base 86: mod_base = OTHER; note = phosphorothioate backbone
  modified_base 87: mod_base = OTHER; note = phosphorothioate backbone
  modified_base 88: mod_base = OTHER; note = phosphorothioate backbone
attacaccttcttccttgacgattacactggcagggctcacatccaaatttttggagcaggttttctgacttcggtcggaaaacccct

SEQ ID NO: 66 - RNA, 97 nt, synthetic construct
  source 1..97: mol_type = other RNA
  modified_base 1: mod_base = OTHER; note = 2'-OME
  modified_base 2: mod_base = OTHER; note = 2'-OME
  modified_base 3: mod_base = um
  modified_base 95: mod_base = cm
  modified_base 96: mod_base = cm
  modified_base 97: mod_base = um
  modified_base 1: mod_base = OTHER; note = phosphorothioate backbone
  modified_base 2: mod_base = OTHER; note = phosphorothioate backbone
  modified_base 3: mod_base = OTHER; note = phosphorothioate backbone
  modified_base 95: mod_base = OTHER; note = phosphorothioate backbone
  modified_base 96: mod_base = OTHER; note = phosphorothioate backbone
  modified_base 97: mod_base = OTHER; note = phosphorothioate backbone
aattacaccttcttccttgacgattaggacactggcagggctcacatccaacatcaatttttggagcaggttttctgacttcggtcggaaaacccct

SEQ ID NO: 67 - DNA, 29 bp, synthetic construct
  source 1..29: mol_type = other DNA
ccgcaatatgatagggacttagggtgnnn

SEQ ID NO: 68 - DNA, 22 bp, synthetic construct
  source 1..22: mol_type = other DNA
caccctaagtccctatcatatt

SEQ ID NO: 69 - DNA, 24 bp, synthetic construct
  source 1..24: mol_type = other DNA
ggttagatgtcaccaattgtaagg

SEQ ID NO: 70 - DNA, 22 bp, synthetic construct
  source 1..22: mol_type = other DNA
aacattgggcttgcagatgcac

SEQ ID NO: 71 - DNA, 17 bp, synthetic construct
  source 1..17: mol_type = other DNA
  modified_base 1: mod_base = OTHER; note = FAM Fluorophore
  modified_base 17: mod_base = OTHER; note = MGB Fluorophore
ctgtcttagcattacag

SEQ ID NO: 72 - DNA, 21 bp, synthetic construct
  source 1..21: mol_type = other DNA
gatggctgcagtccctgtaac

SEQ ID NO: 73 - DNA, 27 bp, synthetic construct
  source 1..27: mol_type = other DNA
gcctggagaaatataaaaaccaataac

SEQ ID NO: 74 - DNA, 16 bp, synthetic construct
  source 1..16: mol_type = other DNA
  modified_base 1: mod_base = OTHER; note = FAM Fluorophore
  modified_base 16: mod_base = OTHER; note = MGB Fluorophore
caatacctctgggaca

SEQ ID NO: 75 - DNA, 53 bp, synthetic construct
  source 1..53: mol_type = other DNA
ccgcaattacaccttcttccttgacgattacactggcagggctcacatccaac

SEQ ID NO: 76 - DNA, 53 bp, synthetic construct
  source 1..53: mol_type = other DNA
aattgttggatgtgagccctgccagtgtaatcgtcaaggaagaaggtgtaatt

SEQ ID NO: 77 - RNA, 21 nt, synthetic construct
  source 1..21: mol_type = other RNA
  modified_base 1..21: mod_base = OTHER; note = 2'-OME
  modified_base 1..21: mod_base = OTHER; note = phosphorothioate
agcttcggagaaatttaaatc

SEQ ID NO: 78 - RNA, 21 nt, synthetic construct
  source 1..21: mol_type = other RNA
  modified_base 1..21: mod_base = OTHER; note = 2'-OME
  modified_base 1..21: mod_base = OTHER; note = phosphorothioate
tgatcacacctaagccctaaa

SEQ ID NO: 79 - RNA, 91 nt, synthetic construct
  source 1..91: mol_type = other RNA
  modified_base 1: mod_base = OTHER; note = 2'-OME
  modified_base 2: mod_base = cm
  modified_base 3: mod_base = cm
  modified_base 89: mod_base = cm
  modified_base 90: mod_base = cm
  modified_base 91: mod_base = um
  modified_base 1: mod_base = OTHER; note = phosphorothioate backbone
  modified_base 2: mod_base = OTHER; note = phosphorothioate backbone
  modified_base 3: mod_base = OTHER; note = phosphorothioate backbone
  modified_base 89: mod_base = OTHER; note = phosphorothioate backbone
  modified_base 90: mod_base = OTHER; note = phosphorothioate backbone
  modified_base 91: mod_base = OTHER; note = phosphorothioate backbone
accgcaatatgatagggacttagggtgacactggcagggctcacatccaaatttttggagcaggttttctgacttcggtcggaaaacccct

SEQ ID NO: 80 - RNA, 93 nt, synthetic construct
  source 1..93: mol_type = other RNA
  modified_base 1: mod_base = OTHER; note = 2'-OME
  modified_base 2: mod_base = cm
  modified_base 3: mod_base = cm
  modified_base 91: mod_base = cm
  modified_base 92: mod_base = cm
  modified_base 93: mod_base = um
  modified_base 1: mod_base = OTHER; note = phosphorothioate backbone
  modified_base 2: mod_base = OTHER; note = phosphorothioate backbone
  modified_base 3: mod_base = OTHER; note = phosphorothioate backbone
  modified_base 91: mod_base = OTHER; note = phosphorothioate backbone
  modified_base 92: mod_base = OTHER; note = phosphorothioate backbone
  modified_base 93: mod_base = OTHER; note = phosphorothioate backbone
accgcaatatgatagggacttagggtgattacaccttcttccttgacgattaatttttggagcaggttttctgacttcggtcggaaaacccct

SEQ ID NO: 81 - DNA, 29 bp, synthetic construct
  source 1..29: mol_type = other DNA
ccgcaatatgatagggacttagggtgnnn

SEQ ID NO: 82 - DNA, 29 bp, synthetic construct
  source 1..29: mol_type = other DNA
aattnnncaccctaagtccctatcatatt